European Patent Application EP 4 631 965 A1, published October 15, 2025. Title: Peptide for cartilage regeneration and uses thereof. Applicant: CAREGEN CO., LTD. The sequence listing filed with the application follows.

SEQUENCE LISTING (14 sequences)

SEQ ID NO: 1 - protein, 5 aa, synthetic construct
PYYRI

SEQ ID NO: 2 - protein, 5 aa, synthetic construct
KFLIK

SEQ ID NO: 3 - DNA, 23 bp, synthetic construct
  source 1..23: mol_type = other DNA
ctatctggacgaagcagctggca

SEQ ID NO: 4 - DNA, 22 bp, synthetic construct
  source 1..22: mol_type = other DNA
atgggtgcaatgtcaatgatgg

SEQ ID NO: 5 - DNA, 20 bp, synthetic construct
  source 1..20: mol_type = other DNA
aactcagggcaggaggatgt

SEQ ID NO: 6 - DNA, 20 bp, synthetic construct
  source 1..20: mol_type = other DNA
tgtccttttggtcgtcgttc

SEQ ID NO: 7 - DNA, 20 bp, synthetic construct
  source 1..20: mol_type = other DNA
ccagcccgaacttgtaaaga

SEQ ID NO: 8 - DNA, 20 bp, synthetic construct
  source 1..20: mol_type = other DNA
tggacgcacaaccatcatac

SEQ ID NO: 9 - DNA, 20 bp, synthetic construct
  source 1..20: mol_type = other DNA
gcaggctatgagcagtgtga

SEQ ID NO: 10 - DNA, 20 bp, synthetic construct
  source 1..20: mol_type = other DNA
gcatacctcggaagcagaag

SEQ ID NO: 11 - DNA, 20 bp, synthetic construct
  source 1..20: mol_type = other DNA
accacagtccatgccatcac

SEQ ID NO: 12 - DNA, 20 bp, synthetic construct
  source 1..20: mol_type = other DNA
tccaccaccctgttgctgta

SEQ ID NO: 13 - DNA, 20 bp, synthetic construct
  source 1..20: mol_type = other DNA
gcggaggaagtcggtgaaga

SEQ ID NO: 14 - DNA, 20 bp, synthetic construct
  source 1..20: mol_type = other DNA
ccctctcgcttcaggtcagc